European Patent Application EP 4 141 118 A1, published March 1, 2023. Title: TECHNIQUE FOR PREPARING UNIVERSAL HUMANISED CAR19-DNT CELLS AND APPLICATION THEREFOR. Applicant: ZHEJIANG RUIJIAMEI BIOTECH CO., LTD. Application PCT/CN2021/087311. The sequence listing filed with the application follows.

SEQUENCE LISTING (16 sequences)

SEQ ID NO: 1 - DNA, 321 bp, artificial sequence
  humanized CD19 VL
gatattcagatgacccagagcccgagcagcctgagcgcgagcgtgggcgatcgcgtgaccattacctgccgcgcgagccaggatattagcaaatatctgaactggtatcagcagaaaccgggcaaagcgccgaaactgctgatttatcataccagccgcctgcatagcggcgtgccgagccgctttagcggcagcggcagcggcaccgattttaccctgaccattagcagcctgcagccggaagattttgcgacctattattgccagcagggcaacaccctgccgtatacctttggcggcggcaccaaagtggaaattaaa

SEQ ID NO: 2 - DNA, 360 bp, artificial sequence
  the nucleotide sequence of VH
caggtgcagctgcaggaaagcggcccgggcctggtgaaaccgagcgaaaccctgagcctgacctgcaccgtgagcggcggcagcctgccggattatggcgtgagctggattcgccagccgccgggcaaaggcctggaatggattggcgtgatttggggcagcgaaaccacctattataacagcgcgctgaaaagccgcgtgaccattagcgtggataccagcaaaaaccagtttagcctgaaactgagcagcgtgaccgcggcggataccgcggtgtattattgcgcgaaacattattattatggcggcagctatgcgatggattattggggccagggcaccctggtgaccgtgagcagc

SEQ ID NO: 3 - DNA, 54 bp, artificial sequence
  the nucleotide sequence
ggctccacctctggatccggcaagcccggatctggcgagggatccaccaagggc

SEQ ID NO: 4 - protein, 245 aa, artificial sequence
  Humanized CD19 scFv
DIQMTQSPSSLSASVGDRVTITCRASQDISKYLNWYQQKPGKAPKLLIYHTSRLHSGVPSRFSGSGSGTDFTLTISSLQPEDFATYYCQQGNTLPYTFGGGTKVEIKGSTSGSGKPGSGEGSTKGQVQLQESGPGLVKPSETLSLTCTVSGGSLPDYGVSWIRQPPGKGLEWIGVIWGSETTYYNSALKSRVTISVDTSKNQFSLKLSSVTAADTAVYYCAKHYYYGGSYAMDYWGQGTLVTVSS

SEQ ID NO: 5 - protein, 107 aa, artificial sequence
  the amino acid sequence of VL
DIQMTQSPSSLSASVGDRVTITCRASQDISKYLNWYQQKPGKAPKLLIYHTSRLHSGVPSRFSGSGSGTDFTLTISSLQPEDFATYYCQQGNTLPYTFGGGTKVEIK

SEQ ID NO: 6 - protein, 120 aa, artificial sequence
  the amino acid sequence of VH
QVQLQESGPGLVKPSETLSLTCTVSGGSLPDYGVSWIRQPPGKGLEWIGVIWGSETTYYNSALKSRVTISVDTSKNQFSLKLSSVTAADTAVYYCAKHYYYGGSYAMDYWGQGTLVTVSS

SEQ ID NO: 7 - protein, 18 aa, artificial sequence
  the amino acid sequence of the linker peptide
GSTSGSGKPGSGEGSTKG

SEQ ID NO: 8 - DNA, 63 bp, artificial sequence
  CD8 leader
atggccttaccagtgaccgccttgctcctgccgctggccttgctgctccacgccgccaggccg

SEQ ID NO: 9 - DNA, 135 bp, artificial sequence
  CD8 Hinge
accacgacgccagcgccgcgaccaccaacaccggcgcccaccatcgcgtcgcagcccctgtccctgcgcccagaggcgtgccggccagcggcggggggcgcagtgcacacgagggggctggacttcgcctgtgat

SEQ ID NO: 10 - DNA, 72 bp, artificial sequence
  CD8 TM
atctacatctgggcgcccctggccgggacttgtggggtccttctcctgtcactggttatcaccctttactgc

SEQ ID NO: 11 - DNA, 126 bp, artificial sequence
  4-1BB Co-stimulated domains
aaacggggcagaaagaaactcctgtatatattcaaacaaccatttatgagaccagtacaaactactcaagaggaagatggctgtagctgccgatttccagaagaagaagaaggaggatgtgaactg

SEQ ID NO: 12 - DNA, 342 bp, artificial sequence
  CD3
agagtgaagttcagcaggagcgcagacgcccccgcgtacaagcagggccagaaccagctctataacgagctcaatctaggacgaagagaggagtacgatgttttggacaagagacgtggccgggaccctgagatggggggaaagccgagaaggaagaaccctcaggaaggcctgtacaatgaactgcagaaagataagatggcggaggcctacagtgagattgggatgaaaggcgagcgccggaggggcaaggggcacgatggcctttaccagggtctcagtacagccaccaaggacacctacgacgcccttcacatgcaggccctgccccctcgctaatag

SEQ ID NO: 13 - DNA, 6 bp, artificial sequence
  EcoRI restriction site
gaattc

SEQ ID NO: 14 - protein, 489 aa, artificial sequence
  humanized CD19-4-1BB-CD3-CAR protein
MALPVTALLLPLALLLHAARPDIQMTQSPSSLSASVGDRVTITCRASQDISKYLNWYQQKPGKAPKLLIYHTSRLHSGVPSRFSGSGSGTDFTLTISSLQPEDFATYYCQQGNTLPYTFGGGTKVEIKGSTSGSGKPGSGEGSTKGQVQLQESGPGLVKPSETLSLTCTVSGGSLPDYGVSWIRQPPGKGLEWIGVIWGSETTYYNSALKSRVTISVDTSKNQFSLKLSSVTAADTAVYYCAKHYYYGGSYAMDYWGQGTLVTVSSTTTPAPRPPTPAPTIASQPLSLRPEACRPAAGGAVHTRGLDFACDIYIWAPLAGTCGVLLLSLVITLYCKRGRKKLLYIFKQPFMRPVQTTQEEDGCSCRFPEEEEGGCELRVKFSRSADAPAYKQGQNQLYNELNLGRREEYDVLDKRRGRDPEMGGKPRRKNPQEGLYNELQKDKMAEAYSEIGMKGERRRGKGHDGLYQGLSTATKDTYDALHMQALPPR

SEQ ID NO: 15 - DNA, 735 bp, artificial sequence
  humanized CD19 (VL-linker-VH), clone 11 scFv
gatattcagatgacccagagcccgagcagcctgagcgcgagcgtgggcgatcgcgtgaccattacctgccgcgcgagccaggatattagcaaatatctgaactggtatcagcagaaaccgggcaaagcgccgaaactgctgatttatcataccagccgcctgcatagcggcgtgccgagccgctttagcggcagcggcagcggcaccgattttaccctgaccattagcagcctgcagccggaagattttgcgacctattattgccagcagggcaacaccctgccgtatacctttggcggcggcaccaaagtggaaattaaaggctccacctctggatccggcaagcccggatctggcgagggatccaccaagggccaggtgcagctgcaggaaagcggcccgggcctggtgaaaccgagcgaaaccctgagcctgacctgcaccgtgagcggcggcagcctgccggattatggcgtgagctggattcgccagccgccgggcaaaggcctggaatggattggcgtgatttggggcagcgaaaccacctattataacagcgcgctgaaaagccgcgtgaccattagcgtggataccagcaaaaaccagtttagcctgaaactgagcagcgtgaccgcggcggataccgcggtgtattattgcgcgaaacattattattatggcggcagctatgcgatggattattggggccagggcaccctggtgaccgtgagcagc

SEQ ID NO: 16 - DNA, 1473 bp, artificial sequence
  The nucleotide sequence of humanized CD19-4-1BB-CD3-CAR protein
atggccttaccagtgaccgccttgctcctgccgctggccttgctgctccacgccgccaggccggatattcagatgacccagagcccgagcagcctgagcgcgagcgtgggcgatcgcgtgaccattacctgccgcgcgagccaggatattagcaaatatctgaactggtatcagcagaaaccgggcaaagcgccgaaactgctgatttatcataccagccgcctgcatagcggcgtgccgagccgctttagcggcagcggcagcggcaccgattttaccctgaccattagcagcctgcagccggaagattttgcgacctattattgccagcagggcaacaccctgccgtatacctttggcggcggcaccaaagtggaaattaaaggctccacctctggatccggcaagcccggatctggcgagggatccaccaagggccaggtgcagctgcaggaaagcggcccgggcctggtgaaaccgagcgaaaccctgagcctgacctgcaccgtgagcggcggcagcctgccggattatggcgtgagctggattcgccagccgccgggcaaaggcctggaatggattggcgtgatttggggcagcgaaaccacctattataacagcgcgctgaaaagccgcgtgaccattagcgtggataccagcaaaaaccagtttagcctgaaactgagcagcgtgaccgcggcggataccgcggtgtattattgcgcgaaacattattattatggcggcagctatgcgatggattattggggccagggcaccctggtgaccgtgagcagcaccacgacgccagcgccgcgaccaccaacaccggcgcccaccatcgcgtcgcagcccctgtccctgcgcccagaggcgtgccggccagcggcggggggcgcagtgcacacgagggggctggacttcgcctgtgatatctacatctgggcgcccctggccgggacttgtggggtccttctcctgtcactggttatcaccctttactgcaaacggggcagaaagaaactcctgtatatattcaaacaaccatttatgagaccagtacaaactactcaagaggaagatggctgtagctgccgatttccagaagaagaagaaggaggatgtgaactgagagtgaagttcagcaggagcgcagacgcccccgcgtacaagcagggccagaaccagctctataacgagctcaatctaggacgaagagaggagtacgatgttttggacaagagacgtggccgggaccctgagatggggggaaagccgagaaggaagaaccctcaggaaggcctgtacaatgaactgcagaaagataagatggcggaggcctacagtgagattgggatgaaaggcgagcgccggaggggcaaggggcacgatggcctttaccagggtctcagtacagccaccaaggacacctacgacgcccttcacatgcaggccctgccccctcgctaatag